European Patent Specification EP 3 362 052 B1, published February 12, 2025. Title: PROCESS FOR PREPARING FORMULATIONS FOR GASTROINTESTINAL-TARGETED THERAPIES. Applicant: Merck Sharp & Dohme Corp. The sequence listing filed with the application follows.

SEQUENCE LISTING (2 sequences)

SEQ ID NO: 1 - protein, 450 aa, Artificial Sequence
  Synthetic Polypeptide
QVQLVQSGAEVKKPGASVKVSCKASGYIFTDYAMHWVRQAPGQGLEWMGTFIPLLDTSDYAQKFQGRVTMTADTSTSTAYMELRSLRSDDTAVYYCARMGVTHSYVMDAWGQGTLVTVSSASTKGPSVFPLAPSSKSTSGGTAALGCLVKDYFPEPVTVSWNSGALTSGVHTFPAVLQSSGLYSLSSVVTVPSSSLGTQTYICNVNHKPSNTKVDKKVEPKSCDKTHTCPPCPAPELLGGPSVFLFPPKPKDTLMISRTPEVTCVVVDVSHEDPEVKFNWYVDGVEVHNAKTKPREEQYNSTYRVVSVLTVLHQDWLNGKEYKCKVSNKALPAPIEKTISKAKGQPREPQVYTLPPSRDELTKNQVSLTCLVKGFYPSDIAVEWESNGQPENNYKTTPPVLDSDGSFFLYSKLTVDKSRWQQGNVFSCSVMHEALHNHYTQKSLSLSPGK

SEQ ID NO: 2 - protein, 214 aa, Artificial Sequence
  Synthetic Polypeptide
EIVLTQSPGTLSLSPGERATLSCRASQPISISVHWYQQKPGQAPRLLIYFASQSISGIPDRFSGSGSGTDFTLTISRLEPEDFAVYYCQQTFSLPYTFGQGTKVEIKRTVAAPSVFIFPPSDEQLKSGTASVVCLLNNFYPREAKVQWKVDNALQSGNSQESVTEQDSKDSTYSLSSTLTLSKADYEKHKVYACEVTHQGLSSPVTKSFNRGEC